European Patent Application EP 4 613 861 A1, published September 10, 2025. Title: EXPRESSION CASSETTE FOR TARGET GENE AND USE THEREOF. Applicant: SUZHOU HEGUANG KEHUI BIOTECHNOLOGY CO., LTD. The sequence listing filed with the application follows.

SEQUENCE LISTING (16 sequences)

SEQ ID NO: 1 - DNA, 1503 bp, synthetic construct
  source 1..1503: mol_type = other DNA; note = Codon-optimized SerpinG1 sequence
atggcttctaggctgacactgctgacactgctgctgctgctgctggctggagatagagcctccagcaatcccaatgccacatccagctccagccaagaccctgagagcctccaagacagaggtgagggcaaagtggccacaactgtgatctccaagatgctctttgtggagcctattctggaggtgagctctctgcccaccaccaattccacaaccaattctgccaccaagatcactgccaacaccactgatgagcctacaacacagcctacaacagaacctaccacacagcccaccattcagcccacccagcccaccacacagctgcctactgacagccctacccagcctaccactggcagcttctgtcctggacctgtgacactgtgctctgatctggagagccatagcacagaggctgtgctgggtgatgctctggtggatttctctctgaagctgtatcatgccttctctgccatgaagaaggtagagacaaacatggcctttagccccttctccattgcttctctgctcacacaagtgctgctgggtgctggtgagaataccaagaccaatctggagtccatcctctcctaccccaaggactttacatgtgtgcaccaagccctcaagggattcaccaccaagggagtgacaagtgtgagccaaatcttccactcccctgacctggccatcagagacacctttgtgaatgcctctaggacactgtacagctcctcccccagagtgctgagcaataatagtgatgccaatctggagctcatcaatacatgggtggctaagaataccaacaacaagatctctaggctgctggattccctcccttctgacacaagactggtgctgctgaatgccatttatctgagtgccaagtggaagaccacatttgaccccaagaagacaagaatggagccctttcacttcaagaactctgtcatcaaggtgcccatgatgaacagtaagaagtatcctgtggcccacttcattgaccagaccctcaaggccaaagtgggacagctgcagctgagccacaatctgtctctggtgattctggtgccccagaatctgaaacatagactggaggacatggaacaagctctgagccccagtgtctttaaggccatcatggagaagctggagatgtccaagttccagcccacactcctcacactgcctagaatcaaagtcaccacaagccaagacatgctgagcatcatggaaaagctggaattctttgacttcagctatgatctgaacctctgtggactcacagaggatcctgatctgcaagtgagtgccatgcagcaccagactgtgctggaactgactgaaactggagtggaggctgctgctgccagtgctatcagtgtggctagaacactgctggtgtttgaggtgcagcagccctttctgtttgtcctctgggatcagcagcataagttccctgtgttcatgggaagggtgtatgatcctagagcctga

SEQ ID NO: 2 - DNA, 1503 bp, Homo sapiens
  source 1..1503: mol_type = other DNA
atggcctccaggctgaccctgctgaccctcctgctgctgctgctggctggggatagagcctcctcaaatccaaatgctaccagctccagctcccaggatccagagagtttgcaagacagaggcgaagggaaggtcgcaacaacagttatctccaagatgctattcgttgaacccatcctggaggtttccagcttgccgacaaccaactcaacaaccaattcagccaccaaaataacagctaataccactgatgaacccaccacacaacccaccacagagcccaccacccaacccaccatccaacccacccaaccaactacccagctcccaacagattctcctacccagcccactactgggtccttctgcccaggacctgttactctctgctctgacttggagagtcattcaacagaggccgtgttgggggatgctttggtagatttctccctgaagctctaccacgccttctcagcaatgaagaaggtggagaccaacatggccttttccccattcagcatcgccagcctccttacccaggtcctgctcggggctggggagaacaccaaaacaaacctggagagcatcctctcttaccccaaggacttcacctgtgtccaccaggccctgaagggcttcacgaccaaaggtgtcacctcagtctctcagatcttccacagcccagacctggccataagggacacctttgtgaatgcctctcggaccctgtacagcagcagccccagagtcctaagcaacaacagtgacgccaacttggagctcatcaacacctgggtggccaagaacaccaacaacaagatcagccggctgctagacagtctgccctccgatacccgccttgtcctcctcaatgctatctacctgagtgccaagtggaagacaacatttgatcccaagaaaaccagaatggaaccctttcacttcaaaaactcagttataaaagtgcccatgatgaatagcaagaagtaccctgtggcccatttcattgaccaaactttgaaagccaaggtggggcagctgcagctctcccacaatctgagtttggtgatcctggtaccccagaacctgaaacatcgtcttgaagacatggaacaggctctcagcccttctgttttcaaggccatcatggagaaactggagatgtccaagttccagcccactctcctaacactaccccgcatcaaagtgacgaccagccaggatatgctctcaatcatggagaaattggaattcttcgatttttcttatgaccttaacctgtgtgggctgacagaggacccagatcttcaggtttctgcgatgcagcaccagacagtgctggaactgacagagactggggtggaggcggctgcagcctccgccatctctgtggcccgcaccctgctggtctttgaagtgcagcagcccttcctcttcgtgctctgggaccagcagcacaagttccctgtcttcatggggcgagtatatgaccccagggcctaa

SEQ ID NO: 3 - DNA, 2677 bp, synthetic construct
  source 1..2677: mol_type = other DNA; note = Y602 expression cassette sequence
taaaatgggcaaacatgctgtttactgagctgggcaccgtaaaatgggcaaacattgcaagcagcaaacagcaaacacacagccctccctgcctgctgaccttggagctggggcagaggtcagagacctctctgggcccatgccacctccaacatccactcgaccccttggaatttcggtggagaggagcagaggttgtcctggcgtggtttaggtagtgtgagagggaggacgccgctgtttactgagctgggcacaatgacctttggcgagctggacagagggccgggcgcagacgggcaggcgggtgggcagctcggcgctgacctttgcccttagtccctgtttgctcctccgataaccggggtgactttggttaatcattaaccagcaaccacccccgtcgtccctgcgggtccacagcttaaatacgaactcgaacggggctctgtctccttagccaggcaccaccactgacctgggacagtgaatcgggctcgcggttgaggacaaactcttcgcggtctttccagtactcttggatcggaaacccgtcggcctccgaacggtactccgccaccgagggacctgagcgagtccgcatcgaccggatcggaaaacctctcgagaaaggcgtctaaccagtcacagtcgcaaggtaggctgagcaccgtggcgggcggcagcgggtggcggtcggggttgtttctggcggaggtgctgctgatgatgtaattaaagtaggcggtcttgagacggcggatggtcgaggtgaggtgtggcaggcttgagatccagctgttggggtgagtactccctctcaaaagcgggcattacttctgcgctaagattgtcagtttccaaaaacgaggaggatttgatattcacctggcccgatctggccatacacttgagtgacaatgacatccactttgcctttctctccacaggtgtccactcccaggtccaagtttaaactctctaaggtaaatataaaatttttaagtgtataatgtgttaaactactgattctaattgtttctctcttttagattccaacctttggaactgagccaccatggcttctaggctgacactgctgacactgctgctgctgctgctggctggagatagagcctccagcaatcccaatgccacatccagctccagccaagaccctgagagcctccaagacagaggtgagggcaaagtggccacaactgtgatctccaagatgctctttgtggagcctattctggaggtgagctctctgcccaccaccaattccacaaccaattctgccaccaagatcactgccaacaccactgatgagcctacaacacagcctacaacagaacctaccacacagcccaccattcagcccacccagcccaccacacagctgcctactgacagccctacccagcctaccactggcagcttctgtcctggacctgtgacactgtgctctgatctggagagccatagcacagaggctgtgctgggtgatgctctggtggatttctctctgaagctgtatcatgccttctctgccatgaagaaggtagagacaaacatggcctttagccccttctccattgcttctctgctcacacaagtgctgctgggtgctggtgagaataccaagaccaatctggagtccatcctctcctaccccaaggactttacatgtgtgcaccaagccctcaagggattcaccaccaagggagtgacaagtgtgagccaaatcttccactcccctgacctggccatcagagacacctttgtgaatgcctctaggacactgtacagctcctcccccagagtgctgagcaataatagtgatgccaatctggagctcatcaatacatgggtggctaagaataccaacaacaagatctctaggctgctggattccctcccttctgacacaagactggtgctgctgaatgccatttatctgagtgccaagtggaagaccacatttgaccccaagaagacaagaatggagccctttcacttcaagaactctgtcatcaaggtgcccatgatgaacagtaagaagtatcctgtggcccacttcattgaccagaccctcaaggccaaagtgggacagctgcagctgagccacaatctgtctctggtgattctggtgccccagaatctgaaacatagactggaggacatggaacaagctctgagccccagtgtctttaaggccatcatggagaagctggagatgtccaagttccagcccacactcctcacactgcctagaatcaaagtcaccacaagccaagacatgctgagcatcatggaaaagctggaattctttgacttcagctatgatctgaacctctgtggactcacagaggatcctgatctgcaagtgagtgccatgcagcaccagactgtgctggaactgactgaaactggagtggaggctgctgctgccagtgctatcagtgtggctagaacactgctggtgtttgaggtgcagcagccctttctgtttgtcctctgggatcagcagcataagttccctgtgttcatgggaagggtgtatgatcctagagcctgattgcatgttaatcaataaaccggttgattcgtttcagttgaactttggtctcctgtgcttatcttatcggtttccatagcaactggttacacatta

SEQ ID NO: 4 - DNA, 192 bp, synthetic construct
  source 1..192: mol_type = other DNA; note = HCR sequence
ccgtaaaatgggcaaacattgcaagcagcaaacagcaaacacacagccctccctgcctgctgaccttggagctggggcagaggtcagagacctctctgggcccatgccacctccaacatccactcgaccccttggaatttcggtggagaggagcagaggttgtcctggcgtggtttaggtagtgtgagaggg

SEQ ID NO: 5 - DNA, 233 bp, synthetic construct
  source 1..233: mol_type = other DNA; note = DSE sequence
aggacgccgctgtttactgagctgggcacaatgacctttggcgagctggacagagggccgggcgcagacgggcaggcgggtgggcagctcggcgctgacctttgcccttagtccctgtttgctcctccgataaccggggtgactttggttaatcattaaccagcaaccacccccgtcgtccctgcgggtccacagcttaaatacgaactcgaacggggctctgtctccttagc

SEQ ID NO: 6 - DNA, 163 bp, synthetic construct
  source 1..163: mol_type = other DNA; note = TPL sequence
gggctcgcggttgaggacaaactcttcgcggtctttccagtactcttggatcggaaacccgtcggcctccgaacggtactccgccaccgagggacctgagcgagtccgcatcgaccggatcggaaaacctctcgagaaaggcgtctaaccagtcacagtcgca

SEQ ID NO: 7 - DNA, 323 bp, synthetic construct
  source 1..323: mol_type = other DNA; note = eMLP sequence
aggtaggctgagcaccgtggcgggcggcagcgggtggcggtcggggttgtttctggcggaggtgctgctgatgatgtaattaaagtaggcggtcttgagacggcggatggtcgaggtgaggtgtggcaggcttgagatccagctgttggggtgagtactccctctcaaaagcgggcattacttctgcgctaagattgtcagtttccaaaaacgaggaggatttgatattcacctggcccgatctggccatacacttgagtgacaatgacatccactttgcctttctctccacaggtgtccactcccaggtccaagtttaaact

SEQ ID NO: 8 - DNA, 93 bp, synthetic construct
  source 1..93: mol_type = other DNA; note = SV40 intron sequence
ctctaaggtaaatataaaatttttaagtgtataatgtgttaaactactgattctaattgtttctctcttttagattccaacctttggaactga

SEQ ID NO: 9 - protein, 738 aa, Adeno-associated dependoparvovirus A
MAADGYLPDWLEDNLSEGIREWWALKPGAPKPKANQQKQDDGRGLVLPGYKYLGPFNGLDKGEPVNAADAAALEHDKAYDQQLQAGDNPYLRYNHADAEFQERLQEDTSFGGNLGRAVFQAKKRVLEPLGLVEEGAKTAPGKKRPVEPSPQRSPDSSTGIGKKGQQPARKRLNFGQTGDSESVPDPQPLGEPPAAPSGVGPNTMAAGGGAPMADNNEGADGVGSSSGNWHCDSTWLGDRVITTSTRTWALPTYNNHLYKQISNGTSGGATNDNTYFGYSTPWGYFDFNRFHCHFSPRDWQRLINNNWGFRPKRLSFKLFNIQVKEVTQNEGTKTIANNLTSTIQVFTDSEYQLPYVLGSAHQGCLPPFPADVFMIPQYGYLTLNNGSQAVGRSSFYCLEYFPSQMLRTGNNFQFTYTFEDVPFHSSYAHSQSLDRLMNPLIDQYLYYLSRTQTTGGTANTQTLGFSQGGPNTMANQAKNWLPGPCYRQQRVSTTTGQNNNSNFAWTAGTKYHLNGRNSLANPGIAMATHKDDEERFFPSNGILIFGKQNAARDNADYSDVMLTSEEEIKTTNPVATEEYGIVADNLQQQNTAPQIGTVNSQGALPGMVWQNRDVYLQGPIWAKIPHTDGNFHPSPLMGGFGLKHPPPQILIKNTPVPADPPTTFNQSKLNSFITQYSTGQVSVEIEWELQKENSKRWNPEIQYTSNYYKSTSVDFAVNTEGVYSEPRPIGTRYLTRNL

SEQ ID NO: 10 - DNA, 321 bp, synthetic construct
  source 1..321: mol_type = other DNA; note = HCR2 sequence
aggctcagaggcacacaggagtttctgggctcaccctgcccccttccaacccctcagttcccatcctccagcagctgtttgtgtgctgcctctgaagtccacactgaacaaacttcagcctactcatgtccctaaaatgggcaaacattgcaagcagcaaacagcaaacacacagccctccctgcctgctgaccttggagctggggcagaggtcagagacctctctgggcccatgccacctccaacatccactcgaccccttggaatttcggtggagaggagcagaggttgtcctggcgtggtttaggtagtgtgagaggg

SEQ ID NO: 11 - DNA, 252 bp, synthetic construct
  source 1..252: mol_type = other DNA; note = TPL2 sequence
gtgagtctatgggacccttgatgttttctttccccttcttttctatggttaagttcatgtcataggaaggggagaagtaacagggtacagggctcgcggttgaggacaaactcttcgcggtctttccagtactcttggatcggaaacccgtcggcctccgaacggtactccgccaccgagggacctgagcgagtccgcatcgaccggatcggaaaacctctcgagaaaggcgtctaaccagtcacagtcgca

SEQ ID NO: 12 - DNA, 122 bp, synthetic construct
  source 1..122: mol_type = other DNA; note = HBB2 intron segment sequence
gttcggcttctggcgtgtgaccggcggctctagagcctctgctaaccatgttcatgccttcttctttttcctacagctcctgggcaacgtgctggttattgtgctgtctcatcattttggca

SEQ ID NO: 13 - DNA, 96 bp, synthetic construct
  source 1..96: mol_type = other DNA; note = PA3 poly(A) sequence
ttgcatgttaatcaataaaccggttgattcgtttcagttgaactttggtctcctgtgcttatcttatcggtttccatagcaactggttacacatta

SEQ ID NO: 14 - DNA, 225 bp, synthetic construct
  source 1..225: mol_type = other DNA; note = BGH poly(A) sequence
ctgtgccttctagttgccagccatctgttgtttgcccctcccccgtgccttccttgaccctggaaggtgccactcccactgtcctttcctaataaaatgaggaaattgcatcgcattgtctgagtaggtgtcattctattctggggggtggggtggggcaggacagcaagggggaggattgggaagacaatagcaggcatgctggggatggggtgggctctatgg

SEQ ID NO: 15 - DNA, 3018 bp, synthetic construct
  source 1..3018: mol_type = other DNA; note = GS1196-016 expression cassette sequence
aggctcagaggcacacaggagtttctgggctcaccctgcccccttccaacccctcagttcccatcctccagcagctgtttgtgtgctgcctctgaagtccacactgaacaaacttcagcctactcatgtccctaaaatgggcaaacattgcaagcagcaaacagcaaacacacagccctccctgcctgctgaccttggagctggggcagaggtcagagacctctctgggcccatgccacctccaacatccactcgaccccttggaatttcggtggagaggagcagaggttgtcctggcgtggtttaggtagtgtgagagggaggacgccgctgtttactgagctgggcacaatgacctttggcgagctggacagagggccgggcgcagacgggcaggcgggtgggcagctcggcgctgacctttgcccttagtccctgtttgctcctccgataaccggggtgactttggttaatcattaaccagcaaccacccccgtcgtccctgcgggtccacagcttaaatacgaactcgaacggggctctgtctccttagccaggcaccaccactgacctgggacagtgaatcgtgagtctatgggacccttgatgttttctttccccttcttttctatggttaagttcatgtcataggaaggggagaagtaacagggtacagggctcgcggttgaggacaaactcttcgcggtctttccagtactcttggatcggaaacccgtcggcctccgaacggtactccgccaccgagggacctgagcgagtccgcatcgaccggatcggaaaacctctcgagaaaggcgtctaaccagtcacagtcgcaaggtaggctgagcaccgtggcgggcggcagcgggtggcggtcggggttgtttctggcggaggtgctgctgatgatgtaattaaagtaggcggtcttgagacggcggatggtcgaggtgaggtgtggcaggcttgagatccagctgttggggtgagtactccctctcaaaagcgggcattacttctgcgctaagattgtcagtttccaaaaacgaggaggatttgatattcacctggcccgatctggccatacacttgagtgacaatgacatccactttgcctttctctccacaggtgtccactcccaggtccaagtttaaactgttcggcttctggcgtgtgaccggcggctctagagcctctgctaaccatgttcatgccttcttctttttcctacagctcctgggcaacgtgctggttattgtgctgtctcatcattttggcaagccaccatggcttctaggctgacactgctgacactgctgctgctgctgctggctggagatagagcctccagcaatcccaatgccacatccagctccagccaagaccctgagagcctccaagacagaggtgagggcaaagtggccacaactgtgatctccaagatgctctttgtggagcctattctggaggtgagctctctgcccaccaccaattccacaaccaattctgccaccaagatcactgccaacaccactgatgagcctacaacacagcctacaacagaacctaccacacagcccaccattcagcccacccagcccaccacacagctgcctactgacagccctacccagcctaccactggcagcttctgtcctggacctgtgacactgtgctctgatctggagagccatagcacagaggctgtgctgggtgatgctctggtggatttctctctgaagctgtatcatgccttctctgccatgaagaaggtagagacaaacatggcctttagccccttctccattgcttctctgctcacacaagtgctgctgggtgctggtgagaataccaagaccaatctggagtccatcctctcctaccccaaggactttacatgtgtgcaccaagccctcaagggattcaccaccaagggagtgacaagtgtgagccaaatcttccactcccctgacctggccatcagagacacctttgtgaatgcctctaggacactgtacagctcctcccccagagtgctgagcaataatagtgatgccaatctggagctcatcaatacatgggtggctaagaataccaacaacaagatctctaggctgctggattccctcccttctgacacaagactggtgctgctgaatgccatttatctgagtgccaagtggaagaccacatttgaccccaagaagacaagaatggagccctttcacttcaagaactctgtcatcaaggtgcccatgatgaacagtaagaagtatcctgtggcccacttcattgaccagaccctcaaggccaaagtgggacagctgcagctgagccacaatctgtctctggtgattctggtgccccagaatctgaaacatagactggaggacatggaacaagctctgagccccagtgtctttaaggccatcatggagaagctggagatgtccaagttccagcccacactcctcacactgcctagaatcaaagtcaccacaagccaagacatgctgagcatcatggaaaagctggaattctttgacttcagctatgatctgaacctctgtggactcacagaggatcctgatctgcaagtgagtgccatgcagcaccagactgtgctggaactgactgaaactggagtggaggctgctgctgccagtgctatcagtgtggctagaacactgctggtgtttgaggtgcagcagccctttctgtttgtcctctgggatcagcagcataagttccctgtgttcatgggaagggtgtatgatcctagagcctgactgtgccttctagttgccagccatctgttgtttgcccctcccccgtgccttccttgaccctggaaggtgccactcccactgtcctttcctaataaaatgaggaaattgcatcgcattgtctgagtaggtgtcattctattctggggggtggggtggggcaggacagcaagggggaggattgggaagacaatagcaggcatgctggggatggggtgggctctatgg

SEQ ID NO: 16 - RNA, 10 nt, synthetic construct
  source 1..10: mol_type = other RNA; note = Kozak sequence
gccaccatgg